European Patent Specification EP 3 288 567 B1, published March 19, 2025. Title: CELL. Applicant: UCL Business PLC. The sequence listing filed with the application follows.

SEQUENCE LISTING (27 sequences)

SEQ ID NO: 1 - protein, 560 aa, Artificial Sequence
  aCD33-Fc-DAP10 CAR (chimeric antigen receptor)
MAVPTQVLGLLLLWLTDARCDIQMTQSPSSLSASVGDRVTITCRASEDIYFNLVWYQQKPGKAPKLLIYDTNRLADGVPSRFSGSGSGTQYTLTISSLQPEDFATYYCQHYKNYPLTFGQGTKLEIKRSGGGGSGGGGSGGGGSGGGGSRSEVQLVESGGGLVQPGGSLRLSCAASGFTLSNYGMHWIRQAPGKGLEWVSSISLNGGSTYYRDSVKGRFTISRDNAKSTLYLQMNSLRAEDTAVYYCAAQDAYTGGYFDYWGQGTLVTVSSMDPAEPKSPDKTHTCPPCPAPPVAGPSVFLFPPKPKDTLMIARTPEVTCVVVDVSHEDPEVKFNWYVDGVEVHNAKTKPREEQYNSTYRVVSVLTVLHQDWLNGKEYKCKVSNKALPAPIEKTISKAKGQPREPQVYTLPPSRDELTKNQVSLTCLVKGFYPSDIAVEWESNGQPENNYKTTPPVLDSDGSFFLYSKLTVDKSRWQQGNVFSCSVMHEALHNHYTQKSLSLSPGKKDPKFWVLVVVGGVLACYSLLVTVAFIIFWVCARPRRSPAQEDGKVYINMPGRG

SEQ ID NO: 2 - protein, 551 aa, Artificial Sequence
  aGD2-Fc-DAP10 CAR
METDTLLLWVLLLWVPGSTGQVQLQESGPGLVKPSQTLSITCTVSGFSLASYNIHWVRQPPGKGLEWLGVIWAGGSTNYNSALMSRLTISKDNSKNQVFLKMSSLTAADTAVYYCAKRSDDYSWFAYWGQGTLVTVSSGGGGSGGGGSGGGGSENQMTQSPSSLSASVGDRVTMTCRASSSVSSSYLHWYQQKSGKAPKVWIYSTSNLASGVPSRFSGSGSGTDYTLTISSLQPEDFATYYCQQYSGYPITFGQGTKVEIKRSDPAEPKSPDKTHTCPPCPAPPVAGPSVFLFPPKPKDTLMIARTPEVTCVVVDVSHEDPEVKFNWYVDGVEVHNAKTKPREEQYNSTYRVVSVLTVLHQDWLNGKEYKCKVSNKALPAPIEKTISKAKGQPREPQVYTLPPSRDELTKNQVSLTCLVKGFYPSDIAVEWESNGQPENNYKTTPPVLDSDGSFFLYSKLTVDKSRWQQGNVFSCSVMHEALHNHYTQKSLSLSPGKKDPKFWVLVVVGGVLACYSLLVTVAFIIFWVCARPRRSPAQEDGKVYINMPGRG

SEQ ID NO: 3 - protein, 23 aa, Artificial Sequence
  DAP10 signalling domain
CARPRRSPAQEDGKVYINMPGRG

SEQ ID NO: 4 - DNA, 1683 bp, Artificial Sequence
  nucleic acid sequence which encodes a CAR, aCD33-Fc-DAP10 CAR
atggccgtgcccactcaggtcctggggttgttgctactgtggcttacagatgccagatgtgacatccagatgacacagtctccatcttccctgtctgcatctgtcggagatcgcgtcaccatcacctgtcgagcaagtgaggacatttattttaatttagtgtggtatcagcagaaaccaggaaaggcccctaagctcctgatctatgatacaaatcgcttggcagatggggtcccatcacggttcagtggctctggatctggcacacagtatactctaaccataagtagcctgcaacccgaagatttcgcaacctattattgtcaacactataagaattatccgctcacgttcggtcaggggaccaagctggaaatcaaaagatctggtggcggagggtcaggaggcggaggcagcggaggcggtggctcgggaggcggaggctcgagatctgaggtgcagttggtggagtctgggggcggcttggtgcagcctggagggtccctgaggctctcctgtgcagcctcaggattcactctcagtaattatggcatgcactggatcaggcaggctccagggaagggtctggagtgggtctcgtctattagtcttaatggtggtagcacttactatcgagactccgtgaagggccgattcactatctccagggacaatgcaaaaagcaccctctaccttcaaatgaatagtctgagggccgaggacacggccgtctattactgtgcagcacaggacgcttatacgggaggttactttgattactggggccaaggaacgctggtcacagtctcgtctatggatcccgccgagcccaaatctcctgacaaaactcacacatgcccaccgtgcccagcacctcccgtggccggcccgtcagtcttcctcttccccccaaaacccaaggacaccctcatgatcgcccggacccctgaggtcacatgcgtggtggtggacgtgagccacgaagaccctgaggtcaagttcaactggtacgtggacggcgtggaggtgcataatgccaagacaaagccgcgggaggagcagtacaacagcacgtaccgtgtggtcagcgtcctcaccgtcctgcaccaggactggctgaatggcaaggagtacaagtgcaaggtctccaacaaagccctcccagcccccatcgagaaaaccatctccaaagccaaagggcagccccgagaaccacaggtgtacaccctgcccccatcccgggatgagctgaccaagaaccaggtcagcctgacctgcctggtcaaaggcttctatcccagcgacatcgccgtggagtgggagagcaatgggcaaccggagaacaactacaagaccacgcctcccgtgctggactccgacggctccttcttcctctacagcaagctcaccgtggacaagagcaggtggcagcaggggaacgtcttctcatgctccgtgatgcatgaggccctgcacaatcactatacccagaaatctctgagtctgagcccaggcaagaaggaccccaagttctgggtcctggtggtggtgggaggcgtgctggcctgttactctctcctggtgaccgtggccttcatcatcttctgggtgtgcgccagaccacggcggagcccagcccaggaggacggcaaggtgtacatcaacatgcccggccgcggctga

SEQ ID NO: 5 - DNA, 1656 bp, Artificial Sequence
  nucleic acid sequence which encodes a CAR, aGD2-Fc-DAP10 CAR
atggagaccgacaccctgctgctgtgggtgctgctgctgtgggtgccaggcagcaccggccaggtgcagctgcaggagtctggcccaggcctggtgaagcccagccagaccctgagcatcacctgcaccgtgagcggcttcagcctggccagctacaacatccactgggtgcggcagcccccaggcaagggcctggagtggctgggcgtgatctgggctggcggcagcaccaactacaacagcgccctgatgagccggctgaccatcagcaaggacaacagcaagaaccaggtgttcctgaagatgagcagcctgacagccgccgacaccgccgtgtactactgcgccaagcggagcgacgactacagctggttcgcctactggggccagggcaccctggtgaccgtgagctctggcggaggcggctctggcggaggcggctctggcggaggcggcagcgagaaccagatgacccagagccccagcagcttgagcgccagcgtgggcgaccgggtgaccatgacctgcagagccagcagcagcgtgagcagcagctacctgcactggtaccagcagaagagcggcaaggccccaaaggtgtggatctacagcaccagcaacctggccagcggcgtgcccagccggttcagcggcagcggcagcggcaccgactacaccctgaccatcagcagcctgcagcccgaggacttcgccacctactactgccagcagtacagcggctaccccatcaccttcggccagggcaccaaggtggagatcaagcggtcggatcccgccgagcccaaatctcctgacaaaactcacacatgcccaccgtgcccagcacctcccgtggccggcccgtcagtcttcctcttccccccaaaacccaaggacaccctcatgatcgcccggacccctgaggtcacatgcgtggtggtggacgtgagccacgaagaccctgaggtcaagttcaactggtacgtggacggcgtggaggtgcataatgccaagacaaagccgcgggaggagcagtacaacagcacgtaccgtgtggtcagcgtcctcaccgtcctgcaccaggactggctgaatggcaaggagtacaagtgcaaggtctccaacaaagccctcccagcccccatcgagaaaaccatctccaaagccaaagggcagccccgagaaccacaggtgtacaccctgcccccatcccgggatgagctgaccaagaaccaggtcagcctgacctgcctggtcaaaggcttctatcccagcgacatcgccgtggagtgggagagcaatgggcaaccggagaacaactacaagaccacgcctcccgtgctggactccgacggctccttcttcctctacagcaagctcaccgtggacaagagcaggtggcagcaggggaacgtcttctcatgctccgtgatgcatgaggccctgcacaatcactatacccagaaatctctgagtctgagcccaggcaagaaggaccccaagttctgggtcctggtggtggtgggaggcgtgctggcctgttactctctcctggtgaccgtggccttcatcatcttctgggtgtgcgccagaccacggcggagcccagcccaggaggacggcaaggtgtacatcaacatgcccggccgcggctga

SEQ ID NO: 6 - protein, 21 aa, Artificial Sequence
  signal peptide
MGTSLLCWMALCLLGADHADG

SEQ ID NO: 7 - protein, 21 aa, Artificial Sequence
  signal peptide derived from IgG1
MSLPVTALLLPLALLLHAARP

SEQ ID NO: 8 - protein, 20 aa, Artificial Sequence
  signal peptide derived from CD8
MAVPTQVLGLLLLWLTDARC

SEQ ID NO: 9 - protein, 37 aa, Artificial Sequence
  co-stimulatory domain, CD28 endodomain
KRSRLLHSDYMNMTPRRPGPTRKHYQPYAPPRDFAAY

SEQ ID NO: 10 - protein, 48 aa, Artificial Sequence
  co-stimulatory domain, CD27 endodomain
QRRKYRSNKGESPVEPAEPCHYSCPREEEGSTIPIQEDYRKPEPACSP

SEQ ID NO: 11 - protein, 42 aa, Artificial Sequence
  co-stimulatory domain, 41BB endodomain
KRGRKKLLYIFKQPFMRPVQTTQEEDGCSCRFPEEEEGGCEL

SEQ ID NO: 12 - protein, 37 aa, Artificial Sequence
  co-stimulatory domain, OX40 endodomain
RRDQRLPPDAHKPPGGGSFRTPIQEEQADAHSTLAKI

SEQ ID NO: 13 - protein, 188 aa, Artificial Sequence
  co-stimulatory domain, CD30 endodomain
HRRACRKRIRQKLHLCYPVQTSQPKLELVDSRPRRSSTQLRSGASVTEPVAEERGLMSQPLMETCHSVGAAYLESLPLQDASPAGGPSSPRDLPEPRVSTEHTNNKIEKIYIMKADTVIVGTVKAELPEGRGLAGPAEPELEEELEADHTPHYPEQETEPPLGSCSDVMLSVEEEGKEDPLPTAASGK

SEQ ID NO: 14 - protein, 13 aa, Artificial Sequence
  co-stimulatory domain, IL2-R endodomain
TWQRRQRKSRRTI

SEQ ID NO: 15 - protein, 195 aa, Artificial Sequence
  co-stimulatory domain, IL7-R endodomain
KKRIKPIVWPSLPDHKKTLEHLCKKPRKNLNVSFNPESFLDCQIHRVDDIQARDEVEGFLQDTFPQQLEESEKQRLGGDVQSPNCPSEDVVITPESFGRDSSLTCLAGNVSACDAPILSSSRSLDCRESGKNGPHVYQDLLLSLGTTNSTLPPPFSLQSGILTLNPVAQGQPILTSLGSNQEEAYVTMSSFYQNQ

SEQ ID NO: 16 - protein, 285 aa, Artificial Sequence
  co-stimulatory domain, IL21-R endodomain
SLKTHPLWRLWKKIWAVPSPERFFMPLYKGCSGDFKKWVGAPFTGSSLELGPWSPEVPSTLEVYSCHPPRSPAKRLQLTELQEPAELVESDGVPKPSFWPTAQNSGGSAYSEERDRPYGLVSIDTVTVLDAEGPCTWPCSCEDDGYPALDLDAGLEPSPGLEDPLLDAGTTVLSCGCVSAGSPGLGGPLGSLLDRLKPPLADGEDWAGGLPWGGRSPGGVSESEAGSPLAGLDMDTFDSGFVGSDCSSPVECDFTSPGDEGPPRSYLRQWVVIPPPLSSPGPQAS

SEQ ID NO: 17 - protein, 45 aa, Artificial Sequence
  co-stimulatory domain, NKp30 endodomain
GSTVYYQGKCLTWKGPRRQLPAVVPAPLPPPCGSSAHLLPPVPGG

SEQ ID NO: 18 - protein, 63 aa, Artificial Sequence
  co-stimulatory domain, NKp44 endodomain
WWGDIWWKTMMELRSLDTQKATCHLQQVTDLPWTSVSSPVEREILYHTVARTKISDDDDEHTL

SEQ ID NO: 19 - protein, 61 aa, Artificial Sequence
  co-stimulatory domain, DNAM-1 (CD226) endodomain
NRRRRRERRDLFTESWDTQKAPNNYRSPISTSQPTNQSMDDTREDIYVNYPTFSRRPKTRV

SEQ ID NO: 20 - protein, 263 aa, Artificial Sequence
  antigen binding domain
METDTLLLWVLLLWVPGSTGQVQLQESGPGLVKPSQTLSITCTVSGFSLASYNIHWVRQPPGKGLEWLGVIWAGGSTNYNSALMSRLTISKDNSKNQVFLKMSSLTAADTAVYYCAKRSDDYSWFAYWGQGTLVTVSSGGGGSGGGGSGGGGSENQMTQSPSSLSASVGDRVTMTCRASSSVSSSYLHWYQQKSGKAPKVWIYSTSNLASGVPSRFSGSGSGTDYTLTISSLQPEDFATYYCQQYSGYPITFGQGTKVEIKRS

SEQ ID NO: 21 - protein, 272 aa, Artificial Sequence
  antigen binding domain
MAVPTQVLGLLLLWLTDARCDIQMTQSPSSLSASVGDRVTITCRASEDIYFNLVWYQQKPGKAPKLLIYDTNRLADGVPSRFSGSGSGTQYTLTISSLQPEDFATYYCQHYKNYPLTFGQGTKLEIKRSGGGGSGGGGSGGGGSGGGGSRSEVQLVESGGGLVQPGGSLRLSCAASGFTLSNYGMHWIRQAPGKGLEWVSSISLNGGSTYYRDSVKGRFTISRDNAKSTLYLQMNSLRAEDTAVYYCAAQDAYTGGYFDYWGQGTLVTVSSM

SEQ ID NO: 22 - protein, 234 aa, Artificial Sequence
  spacer sequence, hinge-CH2CH3 of human IgG1
AEPKSPDKTHTCPPCPAPPVAGPSVFLFPPKPKDTLMIARTPEVTCVVVDVSHEDPEVKFNWYVDGVEVHNAKTKPREEQYNSTYRVVSVLTVLHQDWLNGKEYKCKVSNKALPAPIEKTISKAKGQPREPQVYTLPPSRDELTKNQVSLTCLVKGFYPSDIAVEWESNGQPENNYKTTPPVLDSDGSFFLYSKLTVDKSRWQQGNVFSCSVMHEALHNHYTQKSLSLSPGKKD

SEQ ID NO: 23 - protein, 46 aa, Artificial Sequence
  spacer sequence, human CD8 stalk
TTTPAPRPPTPAPTIASQPLSLRPEACRPAAGGAVHTRGLDFACDI

SEQ ID NO: 24 - protein, 20 aa, Artificial Sequence
  spacer sequence, human IgG1 hinge
AEPKSPDKTHTCPPCPKDPK

SEQ ID NO: 25 - protein, 27 aa, Artificial Sequence
  CD28 transmembrane domain
FWVLVVVGGVLACYSLLVTVAFIIFWV

SEQ ID NO: 26 - protein, 114 aa, Artificial Sequence
  CD3 zeta endodomain
RSRVKFSRSADAPAYQQGQNQLYNELNLGRREEYDVLDKRRGRDPEMGGKPRRKNPQEGLYNELQKDKMAEAYSEIGMKGERRRGKGHDGLYQGLSTATKDTYDALHMQALPPR

SEQ ID NO: 27 - protein, 4 aa, Artificial Sequence
  activation motif
  misc_feature (2)..(3): Xaa can be any naturally occurring amino acid
YXXM